European Patent Application EP 4 606 883 A1, published August 27, 2025. Title: 短柄镰刀菌在生产菌丝体蛋白中的应用. Applicant: 江西富祥生物科技有限公司. The sequence listing filed with the application follows.

SEQUENCE LISTING (6 sequences)

SEQ ID NO: 1 - DNA, 20 bp, synthetic construct
  source 1..20: mol_type = other DNA
atgggtaaggargacaagac

SEQ ID NO: 2 - DNA, 19 bp, synthetic construct
  source 1..19: mol_type = other DNA
ggargtaccagtsatcatg

SEQ ID NO: 3 - DNA, 22 bp, synthetic construct
  source 1..22: mol_type = other DNA
ggaagtaaaagtcgtaacaagg

SEQ ID NO: 4 - DNA, 19 bp, synthetic construct
  source 1..19: mol_type = other DNA
ggtccgtgtttcaagacgg

SEQ ID NO: 5 - DNA, 612 bp, synthetic construct
  source 1..612: mol_type = other DNA
gactctggcaagtcgaccactgtaagtaccaccaagcctcgaccccgcctagatttggtggggtagtctcaagattcatccatactgacatactttgatagaccggtcacttgatctaccagtgcggtggtatcgacaagcgaaccatcgagaagttcgagaaggttggtctcatttccctcgatcgcgcgcccttttacccatcgatccatcattcgactcgctctctcacgacgactcgatccgcgcccgttaccccgctcgagctcaaaaattttgcgaatcaatcgtaatttttttcttgatggggctcataccccgccactcgagtgacgggcgcgcttgccctcttcccacagtcatattcatatgggcgcgcatcatcacgtgtctaccagtcactaaccacttgacaataggaagccgccgagctcggtaagggttccttcaagtacgcctgggttcttgacaagctcaaggccgagcgtgagcgtggtatcaccattgatatcgctctctggaagttcgagactcctcgctactatgtcaccgtcattggtatgctgtcaccgttgccttcatcacatcctcatactaacacgtccaccagac

SEQ ID NO: 6 - DNA, 1065 bp, synthetic construct
  source 1..1065: mol_type = other DNA
ccgagtttacaactcccaaacccctgtgaacatacctttatgttgcctcggcggatcagcccgcgccccgtaaaacgggacggcccgccgcaggaaccacaaaactctgattttagtgtaacttctgagtctaaaaaacaaataaatcaaaactttcaacaacggatctcttggttctggcatcgatgaagaacgcagcaaaatgcgataagtaatgtgaattgcagaattcagtgaatcatcgaatctttgaacgcacattgcgcccgccagtattctggcgggcatgcctgttcgagcgtcatttcaaccctcaagcccccgggtttggtgttggggatcgggctgtactccagcccggccccgaaatctagtggcggtctcgctgcagcctccattgcgtagtagctaacacctcgcaactggaacgcggcgcggccaagccgttaaacccccaacttctgaatgttgacctcggatcaggtaggaatacccgctgaacttaagcatatcaataagcggaggaaaagaaaccaacagggattgccctagtaacggcgagtgaagcggcaacagctcaaatttgaaatctggctctcgggcccgagttgtaatttgtagaggatgcttttgatgcggtgccttccgagttccctggaacgggacgccatagagggtgagagccccgtctggttggatgccaaatctctgtaaagctccttcgacgagtcgagtagtttgggaatgctgctctaaatgggaggtatatgtcttctaaagctaaataccggccagagaccgatagcgcacaagtagagtgatcgaaagatgaaaagcactttgaaaagagagttaaaaagtacgtgaaattgttgaaagggaagcgtttatgaccagacttgggcttggttaatcatctggggttctccccagtgcacttttccagtccaggccagcatcagttttcgccgggggataaaggcttcgggaatgtggctccctccggggagtgttatagcccgttgcgtaataccctggcggggactgaggttcgcgcttctgcaa